European Patent Specification EP 3 342 876 B1, published January 31, 2024. Title: COMPOSITIONS AND METHODS FOR DETECTING GASTROINTESTINAL PATHOGEN NUCLEIC ACID. Applicant: Gen-Probe Prodesse, Inc. Tyler, Ejan. The sequence listing filed with the application follows.

SEQUENCE LISTING (98 sequences)

SEQ ID NO: 1 - DNA, 22 bp, Artificial Sequence
  Synthetic Oligonucleotide
ttatcaagagatgaatgccttc

SEQ ID NO: 2 - DNA, 22 bp, Artificial Sequence
  Synthetic Oligonucleotide
atgttttgtagcatagccgttt

SEQ ID NO: 3 - DNA, 27 bp, Artificial Sequence
  Synthetic Oligonucleotide
ctgctcaaaagaaacaaaagccgaatc

SEQ ID NO: 4 - DNA, 20 bp, Artificial Sequence
  Synthetic Oligonucleotide
ttcttatttggtcccgacag

SEQ ID NO: 5 - DNA, 24 bp, Artificial Sequence
  Synthetic Oligonucleotide
ttgataaatgctatctttaagcgt

SEQ ID NO: 6 - DNA, 22 bp, Artificial Sequence
  Synthetic Oligonucleotide
acgggtgtggtttcgttgagtg

SEQ ID NO: 7 - DNA, 23 bp, Artificial Sequence
  Synthetic Oligonucleotide
cagaagaggctgactcaggaagc

SEQ ID NO: 8 - DNA, 21 bp, Artificial Sequence
  Synthetic Oligonucleotide
ctgaaacgcttaaagatagca

SEQ ID NO: 9 - DNA, 21 bp, Artificial Sequence
  Synthetic Oligonucleotide
aactaataccccgtttaaagc

SEQ ID NO: 10 - DNA, 25 bp, Artificial Sequence
  Synthetic Oligonucleotide
tgcccggttcaacttttgctaacat

SEQ ID NO: 11 - DNA, 29 bp, Artificial Sequence
  Synthetic Oligonucleotide
ttatcaagagatgaatgccttcaaagatc

SEQ ID NO: 12 - DNA, 24 bp, Artificial Sequence
  Synthetic Oligonucleotide
caaaacatgttagcaaaagttgaa

SEQ ID NO: 13 - DNA, 20 bp, Artificial Sequence
  Synthetic Oligonucleotide
tcaccagtcaattgcctctt

SEQ ID NO: 14 - DNA, 24 bp, Artificial Sequence
  Synthetic Oligonucleotide
tccccgcccgataaaataatctcc

SEQ ID NO: 15 - DNA, 28 bp, Artificial Sequence
  Synthetic Oligonucleotide
tatgaggctttaaacggggtattagttg

SEQ ID NO: 16 - DNA, 20 bp, Artificial Sequence
  Synthetic Oligonucleotide
agcctcttctgaaacgctta

SEQ ID NO: 17 - DNA, 20 bp, Artificial Sequence
  Synthetic Oligonucleotide
taccccgtttaaagcctcat

SEQ ID NO: 18 - DNA, 20 bp, Artificial Sequence
  Synthetic Oligonucleotide
gatgcattctaccaacgact

SEQ ID NO: 19 - DNA, 21 bp, Artificial Sequence
  Synthetic Oligonucleotide
tggcgcttcctgagtcagcct

SEQ ID NO: 20 - DNA, 22 bp, Artificial Sequence
  Synthetic Oligonucleotide
aaattcattctcttcacggctt

SEQ ID NO: 21 - DNA, 18 bp, Artificial Sequence
  Synthetic Oligonucleotide
ctgggcagggaaatgttc

SEQ ID NO: 22 - DNA, 23 bp, Artificial Sequence
  Synthetic Oligonucleotide
agtgcggaggtcatttgctgtca

SEQ ID NO: 23 - DNA, 22 bp, Artificial Sequence
  Synthetic Oligonucleotide
tctggaggacattgcccgggat

SEQ ID NO: 24 - DNA, 26 bp, Artificial Sequence
  Synthetic Oligonucleotide
agtcagaactctccattttgtggatg

SEQ ID NO: 25 - DNA, 25 bp, Artificial Sequence
  Synthetic Oligonucleotide
acacgccatagaaacgcatttcctt

SEQ ID NO: 26 - DNA, 20 bp, Artificial Sequence
  Synthetic Oligonucleotide
acgccatagaaacgcatttc

SEQ ID NO: 27 - DNA, 24 bp, Artificial Sequence
  Synthetic Oligonucleotide
agctgaagtttctctgcgagcatg

SEQ ID NO: 28 - DNA, 18 bp, Artificial Sequence
  Synthetic Oligonucleotide
gccgtgaaggaaatgcgt

SEQ ID NO: 29 - DNA, 23 bp, Artificial Sequence
  Synthetic Oligonucleotide
tctatggcgtgtcgggagtgaca

SEQ ID NO: 30 - DNA, 20 bp, Artificial Sequence
  Synthetic Oligonucleotide
tgaagtttctctgcgagcat

SEQ ID NO: 31 - DNA, 18 bp, Artificial Sequence
  Synthetic Oligonucleotide
tgtcgcgctcacatggaa

SEQ ID NO: 32 - DNA, 25 bp, Artificial Sequence
  Synthetic Oligonucleotide
tctggaaggccaggtagacttctat

SEQ ID NO: 33 - DNA, 28 bp, Artificial Sequence
  Synthetic Oligonucleotide
ccacaaaatggagagttctgactttatc

SEQ ID NO: 34 - DNA, 23 bp, Artificial Sequence
  Synthetic Oligonucleotide
tccggaaaaccctcctggtccat

SEQ ID NO: 35 - DNA, 26 bp, Artificial Sequence
  Synthetic Oligonucleotide
cttttcgataatgataccggcgctct

SEQ ID NO: 36 - DNA, 18 bp, Artificial Sequence
  Synthetic Oligonucleotide
acagctctcagtggcatc

SEQ ID NO: 37 - DNA, 18 bp, Artificial Sequence
  Synthetic Oligonucleotide
cttgaccgcctttccgat

SEQ ID NO: 38 - DNA, 23 bp, Artificial Sequence
  Synthetic Oligonucleotide
attccgtgaacaggtcgctgcat

SEQ ID NO: 39 - DNA, 23 bp, Artificial Sequence
  Synthetic Oligonucleotide
aagactgctgtcgaagctccgca

SEQ ID NO: 40 - DNA, 23 bp, Artificial Sequence
  Synthetic Oligonucleotide
tctctgcacgcaatacctccgga

SEQ ID NO: 41 - DNA, 18 bp, Artificial Sequence
  Synthetic Oligonucleotide
gcgccggtatcattatcg

SEQ ID NO: 42 - DNA, 18 bp, Artificial Sequence
  Synthetic Oligonucleotide
caatacctccggattccg

SEQ ID NO: 43 - DNA, 23 bp, Artificial Sequence
  Synthetic Oligonucleotide
ctgatggaccaggagggttttcc

SEQ ID NO: 44 - DNA, 23 bp, Artificial Sequence
  Synthetic Oligonucleotide
ctggaaaaactcagtgcctctgc

SEQ ID NO: 45 - DNA, 18 bp, Artificial Sequence
  Synthetic Oligonucleotide
gcttccgtacgcttcagt

SEQ ID NO: 46 - DNA, 20 bp, Artificial Sequence
  Synthetic Oligonucleotide
aatgcgtttctatggcgtgt

SEQ ID NO: 47 - DNA, 25 bp, Artificial Sequence
  Synthetic Oligonucleotide
cattctcttcacggcttctgaccat

SEQ ID NO: 48 - DNA, 21 bp, Artificial Sequence
  Synthetic Oligonucleotide
atgccatggtccccagaggga

SEQ ID NO: 49 - DNA, 23 bp, Artificial Sequence
  Synthetic Oligonucleotide
tgacagcaaatgacctccgcact

SEQ ID NO: 50 - DNA, 26 bp, Artificial Sequence
  Synthetic Oligonucleotide
atggtcagaagccgtgaagagaatga

SEQ ID NO: 51 - DNA, 22 bp, Artificial Sequence
  Synthetic Oligonucleotide
atgtaattgctgcaaaagcagt

SEQ ID NO: 52 - DNA, 20 bp, Artificial Sequence
  Synthetic Oligonucleotide
ccaagagctaaatctgcatc

SEQ ID NO: 53 - DNA, 27 bp, Artificial Sequence
  Synthetic Oligonucleotide
tcttagcgatgagtggaaagtttatgc

SEQ ID NO: 54 - DNA, 26 bp, Artificial Sequence
  Synthetic Oligonucleotide
aggtgattatccgttccatcgctaac

SEQ ID NO: 55 - DNA, 20 bp, Artificial Sequence
  Synthetic Oligonucleotide
ggctttgattaatccaggtg

SEQ ID NO: 56 - DNA, 22 bp, Artificial Sequence
  Synthetic Oligonucleotide
aattcttccatcaagttctacg

SEQ ID NO: 57 - DNA, 25 bp, Artificial Sequence
  Synthetic Oligonucleotide
ccgaagaacttacttttgcaccatg

SEQ ID NO: 58 - DNA, 27 bp, Artificial Sequence
  Synthetic Oligonucleotide
aggaatggatttaagtcatggtggaca

SEQ ID NO: 59 - DNA, 22 bp, Artificial Sequence
  Synthetic Oligonucleotide
ctttacctgaagtaatggaagt

SEQ ID NO: 60 - DNA, 20 bp, Artificial Sequence
  Synthetic Oligonucleotide
atcaaagccgcataaacacc

SEQ ID NO: 61 - DNA, 27 bp, Artificial Sequence
  Synthetic Oligonucleotide
tgattagcttgagaacctgaattaggc

SEQ ID NO: 62 - DNA, 24 bp, Artificial Sequence
  Synthetic Oligonucleotide
attgtaaatttgctaatgttcagc

SEQ ID NO: 63 - DNA, 22 bp, Artificial Sequence
  Synthetic Oligonucleotide
gaagaacttacttttgcaccat

SEQ ID NO: 64 - DNA, 26 bp, Artificial Sequence
  Synthetic Oligonucleotide
agctaatcaaggtgtttatgcggctt

SEQ ID NO: 65 - DNA, 28 bp, Artificial Sequence
  Synthetic Oligonucleotide
taattcaggttctcaagctaatcaaggt

SEQ ID NO: 66 - DNA, 22 bp, Artificial Sequence
  Synthetic Oligonucleotide
tatggtggttgtgaatttgttg

SEQ ID NO: 67 - DNA, 22 bp, Artificial Sequence
  Synthetic Oligonucleotide
ccatgacttaaatccattccta

SEQ ID NO: 68 - DNA, 27 bp, Artificial Sequence
  Synthetic Oligonucleotide
acctggattaatcaaagccgcataaac

SEQ ID NO: 69 - DNA, 28 bp, Artificial Sequence
  Synthetic Oligonucleotide
ccttgattagcttgagaacctgaattag

SEQ ID NO: 70 - DNA, 30 bp, Artificial Sequence
  Synthetic Oligonucleotide
tgagattgaaactctagctattgaaagatg

SEQ ID NO: 71 - DNA, 21 bp, Artificial Sequence
  Synthetic Oligonucleotide
caaagagttagagcgtcaatg

SEQ ID NO: 72 - DNA, 22 bp, Artificial Sequence
  Synthetic Oligonucleotide
gctagagtttcaatctcatcaa

SEQ ID NO: 73 - DNA, 30 bp, Artificial Sequence
  Synthetic Oligonucleotide
aaggtcttgaaatgatagcgagtgaaaatt

SEQ ID NO: 74 - DNA, 30 bp, Artificial Sequence
  Synthetic Oligonucleotide
aaattcacaaccaccataatatcttttacc

SEQ ID NO: 75 - DNA, 20 bp, Artificial Sequence
  Synthetic Oligonucleotide
agtttgtggagctagtgctt

SEQ ID NO: 76 - DNA, 22 bp, Artificial Sequence
  Synthetic Oligonucleotide
gcaatatgtgctatatcagcaa

SEQ ID NO: 77 - DNA, 31 bp, Artificial Sequence
  Synthetic Oligonucleotide
caagagtgattgattttgctaaatttagaga

SEQ ID NO: 78 - DNA, 20 bp, Artificial Sequence
  Synthetic Oligonucleotide
gatgcagatttagctcttgg

SEQ ID NO: 79 - DNA, 22 bp, Artificial Sequence
  Synthetic Oligonucleotide
tctttaaaacctctggcagtaa

SEQ ID NO: 80 - DNA, 27 bp, Artificial Sequence
  Synthetic Oligonucleotide
tggagttccaagtcttaatccacttgt

SEQ ID NO: 81 - DNA, 29 bp, Artificial Sequence
  Synthetic Oligonucleotide
aatgcaggtattactgcaaataaaaatac

SEQ ID NO: 82 - DNA, 22 bp, Artificial Sequence
  Synthetic Oligonucleotide
caggtttaaaatttcgccttag

SEQ ID NO: 83 - DNA, 22 bp, Artificial Sequence
  Synthetic Oligonucleotide
caaagttgaaacccaactatga

SEQ ID NO: 84 - DNA, 29 bp, Artificial Sequence
  Synthetic Oligonucleotide
caagagatcaaatttctttccatgatgca

SEQ ID NO: 85 - DNA, 29 bp, Artificial Sequence
  Synthetic Oligonucleotide
ctgcatcatggaaagaaatttgatctctt

SEQ ID NO: 86 - DNA, 18 bp, Artificial Sequence
  Synthetic Oligonucleotide
tgctccagctcctgtagt

SEQ ID NO: 87 - DNA, 24 bp, Artificial Sequence
  Synthetic Oligonucleotide
tgattgtatgatctagaacctata

SEQ ID NO: 88 - DNA, 27 bp, Artificial Sequence
  Synthetic Oligonucleotide
cacaatcaaaatgtcctgaagaaccaa

SEQ ID NO: 89 - DNA, 25 bp, Artificial Sequence
  Synthetic Oligonucleotide
agagggtgctttgttggatgagaat

SEQ ID NO: 90 - DNA, 29 bp, Artificial Sequence
  Synthetic Oligonucleotide
tatcagtatgaccctctaaaatagtatca

SEQ ID NO: 91 - DNA, 18 bp, Artificial Sequence
  Synthetic Oligonucleotide
gaaagacgcgctaacagc

SEQ ID NO: 92 - DNA, 19 bp, Artificial Sequence
  Synthetic Oligonucleotide
gagcgtggcttatcttgac

SEQ ID NO: 93 - DNA, 28 bp, Artificial Sequence
  Synthetic Oligonucleotide
ttcggtgtagataaaagtcgtatccaga

SEQ ID NO: 94 - DNA, 27 bp, Artificial Sequence
  Synthetic Oligonucleotide
caactgtctggatacgacttttatcta

SEQ ID NO: 95 - DNA, 459 bp, Salmonella enterica subsp. enterica serovar Typhimurium str. LT2
  ref <308>: AE006468 GI 16445344
  ref <309>: 2011-11-21
  ref <313>: (1)..(459)
tcaccagtcaattgcctctttgttttccccgcccgataaaataatctcctgcatccaggaggtcatttgtgactgtgcgttcattgaaccaactaataccccgtttaaagcctcatataaatgggtgcccggttcaacttttgctaacatgttttgtagcatagccgtttgctgctcaaaagaaacaaaagccgaatcaccactgttaggatctttgaaggcattcatctcttgataaatgctatctttaagcgtttcagaagaggctgactcaggaagcgccaaaagtcgttggtagaatgcatcataaagatcaacgtcgccgccattgcttaaaggcgcgctatccatattattcagcatagcggccctggcactcaacgaaaccacacccgtcgcttcagtatctgctgtcgggaccaaataagaagtcggaatcgtacccggtatcaccttata

SEQ ID NO: 96 - DNA, 1698 bp, Shigella sonnei Ss046 plasmid pSS_046
  ref <308>: CP000039.1  GI:73858315
  ref <309>: 2007-07-30
  ref <313>: (1)..(1698)
atgttctctgtaaataatacacactcatcagtttcttgctccccctctattaactcaaactcaaccagtaatgaatattatctgagaatcctgactgaatgggaaaagaactcttctcccggggaagagcgaggcattgcttttaacagactctcccagtgctttcagaatcaagaagcagtattaaatttatcagacctaaatttgacgtctcttcccgaattaccaaagcatatttctgctttgattgtagaaaataataaattaacatcattgccaaagctgcctgcatttctcaaagaacttaatgctgataataacaggctttctgtgataccagaacttcctgagtcattaacaactttaagtgttcgttctaatcaactggaaaaccttcctgttttgccaaaccatttaacatcattatttgttgaaaataacaggctatataacttaccggctcttcccgaaaaattgaaatttttacatgtttattataacaggctgacaacattacccgacttaccggataaactggaaattctctgtgctcagcgcaataatctggttacttttcctcaattttctgatagaaacaatatcagacaaaaggaatattattttcattttaatcagataaccactcttccggagagtttttcacaattagattcaagttacaggattaatatttcagggaatccattgtcgactcgcgttctgcaatccctgcaaagattaacctcttcgccggactaccacggcccgcagatttacttctccatgagtgacggacaacagaatacactccatcgccccctggctgatgccgtgacagcatggttcccggaaaacaaacaatctgatgtatcacagatatggcatgcttttgaacatgaagagcatgccaacaccttttccgcgttccttgaccgcctttccgataccgtctctgcacgcaatacctccggattccgtgaacaggtcgctgcatggctggaaaaactcagtgcctctgcggagcttcgacagcagtctttcgctgttgctgctgatgccactgagagctgtgaggaccgtgtcgcgctcacatggaacaatctccggaaaaccctcctggtccatcaggcatcagaaggccttttcgataatgataccggcgctctgctctccctgggcagggaaatgttccgcctcgaaattctggaggacattgcccgggataaagtcagaactctccattttgtggatgagatagaagtctacctggccttccagaccatgctcgcagagaaacttcagctctccactgccgtgaaggaaatgcgtttctatggcgtgtcgggagtgacagcaaatgacctccgcactgccgaagccatggtcagaagccgtgaagagaatgaatttacggactggttctccctctggggaccatggcatgctgtactgaagcgtacggaagctgaccgctgggcgcaggcagaagagcagaagtatgagatgctggagaatgagtactctcagagggtggctgaccggctgaaagcatcaggtctgagcggtgatgcggatgcggagagggaagccggtgcacaggtgatgcgtgagactgaacagcagatttaccgtcagttgactgacgaggtactggccctgcgattgtctgaaaacggctcacgactgcaccattcataa

SEQ ID NO: 97 - DNA, 1245 bp, Campylobacter jejuni subsp. jejuni 81116
  ref <308>: CP000814.1  GI:157385286
  ref <309>: 2008-04-23
  ref <313>: (1)..(1245)
atgagtttagaaatgtttgataaagaaatttttgatttaacaaacaaagagttagagcgtcaatgcgaaggtcttgaaatgatagcgagtgaaaatttcactttacctgaagtaatggaagttataggaagtatcttgacgaacaaatacgcagaaggttatccaggtaaaagatattatggtggttgtgaatttgttgatgagattgaaactctagctattgaaagatgtaaaaaactttttaattgtaaatttgctaatgttcagcctaattcaggttctcaagctaatcaaggtgtttatgcggctttgattaatccaggtgataaaattttaggaatggatttaagtcatggtggacatttaactcatggtgcaaaagtaagttcttcgggtaaaatgtacgaaagttgtttttacggcgtagaacttgatggaagaattgattatgaaaaagtaagagaaatcgctaagaaagaaaagccaaaattaatagtttgtggagctagtgcttatgcaagagtgattgattttgctaaatttagagaaattgctgatgaaataggtgcctatctttttgctgatatagcacatattgcaggtcttgttgtggcaggcgagcatccaagtccttttccgcacgctcatgtagtaagctcaaccacacataaaactttgcgtggtccaagaggtggtattattatgacaaatgatgaagagcttgctaaaaaaattaattctgccatttttccaggtattcaaggtggtcctttgatgcatgtaattgctgcaaaagcagtaggatttaaatttaatcttagcgatgagtggaaagtttatgcaaaacaagtaagaaccaatgctcaagttttagctaatgttttaatggatagaaaatttaaacttgttagcgatggaacggataatcaccttgttttaatgagttttttagatcgtgaatttagtggaaaagatgcagatttagctcttggaaatgcaggtattactgcaaataaaaataccgttccaggagagattagaagtccttttatcacaagtggattaagacttggaactccagcgcttactgccagaggttttaaagaaaaagaaatggaaattgtgtcaaattatattgcagatattttagatgatattaataatgaaaaattacaagagaatattaaacaagaattaaaaaaacttgcaagtaattttattatttatgaaagggctatgttttga

SEQ ID NO: 98 - DNA, 673 bp, Campylobacter coli
  gene (1)..(673): Campylobacter coli strain 313 fibronectin-binding protein (cadF) gene, partial sequence.
  ref <308>: FJ946045.1  GI:228018132
  ref <309>: 2010-04-30
  ref <313>: (1)..(673)
cattgatttaggtgagaaattttatttttatggtttagctggtgggggatatgaggatttttctaaaggcgcttttgataataaaagtggaggatttggccattatggagcaggtttaaaatttcgccttagtgattctttagctttaagacttgaaacaagagatcaaatttctttccatgatgcagatcatagttgggtttcaactttgggtattagttttggttttggcgctaagcaagaaaaagttgtagtggagcaaacaaaagaagtagttaataaacctcaagttgtaacccctgctccagctcctgtagtctcacaatcaaaatgtcctgaagaaccaagagagggtgctttgttggatgagaatggttgcgaaaaaacaatttatttagagggacattttgattttgataaagtaaatatcaacccagcctttgaagaacaaatcaaagaaattgctcaaattttagatgaaaatgtaagatatgatactattttagagggtcatactgataatataggttctagatcatacaatcaaaaactttcagaaagacgcgctaacagcgttgcaaaagagcttgaaaaattcggtgtagataaaagtcgtatccagacagttggttatggtcaagataagccacgctcaagcaatgacactaaagag